European Patent Application EP 4 324 841 A1, published February 21, 2024. Title: Cell Penetrating Peptide, Anticancer peptide and Pharmaceutical Composition for Preventing or Treating Cancer comprising the same. Applicant: Onecuregen Co., Ltd. Korea Research Institute of Bioscience and Biotechnology ICURE BNP Co., Ltd. The sequence listing filed with the application follows.

SEQUENCE LISTING (67 sequences)

SEQ ID NO: 1 - protein, 5 aa, Artificial Sequence
  formula1
  UNSURE (1): Arg, Lys, Ala, Val, Ile, Leu, Met, Phe, Tyr or Trp
  UNSURE (2): Arg, Lys or His
  UNSURE (3): Arg or Leu
  UNSURE (4): Arg, Lys, His, Asp, Glu, Ser, Thr, Asn or Gln
  UNSURE (5): Arg, Lys or Val
XXXXX

SEQ ID NO: 2 - protein, 7 aa, Artificial Sequence
  linear peptide
YSSPWTK

SEQ ID NO: 3 - protein, 9 aa, Artificial Sequence
  cyclic peptide
  DISULFID (1)..(9)
CYSSPWTKC

SEQ ID NO: 4 - protein, 11 aa, Artificial Sequence
  Con
YGRKKRRQRRR

SEQ ID NO: 5 - protein, 18 aa, Artificial Sequence
  7
YGRKKRRQRRRYSSPWTK

SEQ ID NO: 6 - protein, 20 aa, Artificial Sequence
  CC
  DISULFID (12)..(20)
YGRKKRRQRRRCYSSPWTKC

SEQ ID NO: 7 - protein, 7 aa, Artificial Sequence
  SII
SIIFRIF

SEQ ID NO: 8 - protein, 12 aa, Artificial Sequence
  OCP1
SIIFRIFLHLQK

SEQ ID NO: 9 - protein, 12 aa, Artificial Sequence
  OCP2
SIIFRIFAHLQK

SEQ ID NO: 10 - protein, 12 aa, Artificial Sequence
  OCP3
SIIFRIFLHLKK

SEQ ID NO: 11 - protein, 12 aa, Artificial Sequence
  OCP4
SIIFRIFAHLKK

SEQ ID NO: 12 - protein, 15 aa, Artificial Sequence
  OCP5
SIIFRIFLHLQKRRR

SEQ ID NO: 13 - protein, 15 aa, Artificial Sequence
  OCP6
SIIFRIFAHLQKRRR

SEQ ID NO: 14 - protein, 15 aa, Artificial Sequence
  OCP7
SIIFRIFLHLKKRRR

SEQ ID NO: 15 - protein, 15 aa, Artificial Sequence
  OCP8
SIIFRIFAHLKKRRR

SEQ ID NO: 16 - protein, 12 aa, Artificial Sequence
  OCP9
SIIFRIFRRRRR

SEQ ID NO: 17 - protein, 14 aa, Artificial Sequence
  OCP10
SIIFRIFRRRRRGD

SEQ ID NO: 18 - protein, 12 aa, Artificial Sequence
  OCP11
RRRRRSIIFRIF

SEQ ID NO: 19 - protein, 12 aa, Artificial Sequence
  OCP12
RRRRRSIIFRGD

SEQ ID NO: 20 - protein, 11 aa, Artificial Sequence
  OCP13
RRRRRGDSIIF

SEQ ID NO: 21 - protein, 14 aa, Artificial Sequence
  OCP14
RRRRRGDSIIFRIF

SEQ ID NO: 22 - protein, 12 aa, Artificial Sequence
  OCP15
KKKKRKVRGDSI

SEQ ID NO: 23 - protein, 15 aa, Artificial Sequence
  OCP16
KKKKRKVSIIFIRGD

SEQ ID NO: 24 - protein, 12 aa, Artificial Sequence
  OCP17
KKKKRKVSIRGD

SEQ ID NO: 25 - protein, 14 aa, Artificial Sequence
  OCP18
KKKKRKVSIIFRIF

SEQ ID NO: 26 - protein, 27 aa, Artificial Sequence
  OCP1-VGLL1S84-15
SIIFRIFLHLQKPNQWRYSSPWTKPQP

SEQ ID NO: 27 - protein, 29 aa, Artificial Sequence
  OCP1-VGLL1S84-15C
  DISULFID (13)..(29)
SIIFRIFLHLQKCPNQWRYSSPWTKPQPC

SEQ ID NO: 28 - protein, 30 aa, Artificial Sequence
  OCP5-VGLL1S84-15
SIIFRIFLHLQKPNQWRYSSPWTKPQPRRR

SEQ ID NO: 29 - protein, 32 aa, Artificial Sequence
  OCP5-VGLL1S84-15C
  DISULFID (13)..(29)
SIIFRIFLHLQKCPNQWRYSSPWTKPQPCRRR

SEQ ID NO: 30 - protein, 19 aa, Artificial Sequence
  OCP1-VGLL1S84-7
SIIFRIFLHLQKYSSPWTK

SEQ ID NO: 31 - protein, 21 aa, Artificial Sequence
  OCP1-VGLL1S84-7C
  DISULFID (13)..(21)
SIIFRIFLHLQKCYSSPWTKC

SEQ ID NO: 32 - protein, 22 aa, Artificial Sequence
  OCP5-VGLL1S84-7
SIIFRIFLHLQKYSSPWTKRRR

SEQ ID NO: 33 - protein, 24 aa, Artificial Sequence
  OCP5-VGLL1S84-7C
  DISULFID (13)..(21)
SIIFRIFLHLQKCYSSPWTKCRRR

SEQ ID NO: 34 - protein, 19 aa, Artificial Sequence
  OCP2-VGLL1S84-7
SIIFRIFAHLQKYSSPWTK

SEQ ID NO: 35 - protein, 21 aa, Artificial Sequence
  OCP2-VGLL1S84-7C
  DISULFID (13)..(21)
SIIFRIFAHLQKCYSSPWTKC

SEQ ID NO: 36 - protein, 19 aa, Artificial Sequence
  OCP3-VGLL1S84-7
SIIFRIFLHLKKYSSPWTK

SEQ ID NO: 37 - protein, 21 aa, Artificial Sequence
  OCP3-VGLL1S84-7C
  DISULFID (13)..(21)
SIIFRIFLHLKKCYSSPWTKC

SEQ ID NO: 38 - protein, 19 aa, Artificial Sequence
  OCP4-VGLL1S84-7
SIIFRIFAHLKKYSSPWTK

SEQ ID NO: 39 - protein, 21 aa, Artificial Sequence
  OCP4-VGLL1S84-7C
  DISULFID (13)..(21)
SIIFRIFAHLKKCYSSPWTKC

SEQ ID NO: 40 - protein, 24 aa, Artificial Sequence
  OCP5-VGLL1S84-7CC
  DISULFID (1)..(24)
CSIIFRIFLHLQKYSSPWTKRRRC

SEQ ID NO: 41 - protein, 26 aa, Artificial Sequence
  OCP5-VGLL1S84-9C
  DISULFID (13)..(23)
SIIFRIFLHLQKCWRYSSPWTKCRRR

SEQ ID NO: 42 - protein, 28 aa, Artificial Sequence
  OCP5-VGLL1S84-11C
  DISULFID (13)..(25)
SIIFRIFLHLQKCNQWRYSSPWTKCRRR

SEQ ID NO: 43 - protein, 19 aa, Artificial Sequence
  OCP9-VGLL1S84-7
SIIFRIFRRRRRYSSPWTK

SEQ ID NO: 44 - protein, 21 aa, Artificial Sequence
  OCP9-VGLL1S84-7CC
  DISULFID (1)..(21)
CSIIFRIFRRRRRYSSPWTKC

SEQ ID NO: 45 - protein, 21 aa, Artificial Sequence
  OCP9-VGLL1S84-9
SIIFRIFRRRRRWRYSSPWTK

SEQ ID NO: 46 - protein, 23 aa, Artificial Sequence
  OCP9-VGLL1S84-9CC
  DISULFID (1)..(23)
CSIIFRIFRRRRRWRYSSPWTKC

SEQ ID NO: 47 - protein, 23 aa, Artificial Sequence
  OCP9-VGLL1S84-11
SIIFRIFRRRRRNQWRYSSPWTK

SEQ ID NO: 48 - protein, 25 aa, Artificial Sequence
  OCP9-VGLL1S84-11CC
  DISULFID (1)..(25)
CSIIFRIFRRRRRNQWRYSSPWTKC

SEQ ID NO: 49 - protein, 27 aa, Artificial Sequence
  OCP9-VGLL1S84-15
SIIFRIFRRRRRPNQWRYSSPWTKPQP

SEQ ID NO: 50 - protein, 29 aa, Artificial Sequence
  OCP9-VGLL1S84-15CC
  DISULFID (1)..(29)
CSIIFRIFRRRRRPNQWRYSSPWTKPQPC

SEQ ID NO: 51 - protein, 23 aa, Artificial Sequence
  OCP10-VGLL1S84-9
SIIFRIFRRRRRGDWRYSSPWTK

SEQ ID NO: 52 - protein, 23 aa, Artificial Sequence
  OCP11-VGLL1S84-11
RRRRRSIIFRIFNQWRYSSPWTK

SEQ ID NO: 53 - protein, 25 aa, Artificial Sequence
  OCP11-VGLL1S84-11CC
  DISULFID (1)..(25)
CRRRRRSIIFRIFNQWRYSSPWTKC

SEQ ID NO: 54 - protein, 23 aa, Artificial Sequence
  OCP12-VGLL1S84-11
RRRRRSIIFRGDNQWRYSSPWTK

SEQ ID NO: 55 - protein, 22 aa, Artificial Sequence
  OCP13-VGLL1S84-11
RRRRRGDSIIFNQWRYSSPWTK

SEQ ID NO: 56 - protein, 25 aa, Artificial Sequence
  OCP14-VGLL1S84-11
RRRRRGDSIIFRIFNQWRYSSPWTK

SEQ ID NO: 57 - protein, 23 aa, Artificial Sequence
  OCP15-VGLL1S84-11
KKKKRKVRGDSINQWRYSSPWTK

SEQ ID NO: 58 - protein, 26 aa, Artificial Sequence
  OCP16-VGLL1S84-11
KKKKRKVSIIFIRGDNQWRYSSPWTK

SEQ ID NO: 59 - protein, 23 aa, Artificial Sequence
  OCP17-VGLL1S84-11
KKKKRKVSIRGDNQWRYSSPWTK

SEQ ID NO: 60 - protein, 25 aa, Artificial Sequence
  OCP18-VGLL1S84-11
KKKKRKVSIIFRIFNQWRYSSPWTK

SEQ ID NO: 61 - DNA, 22 bp, Artificial Sequence
  MMP1_foward
atgaagcagcccagatgtggag

SEQ ID NO: 62 - DNA, 22 bp, Artificial Sequence
  MMP1_reverse
tggtccacatctgctcttggca

SEQ ID NO: 63 - DNA, 20 bp, Artificial Sequence
  MMP9_foward
gggacgcagacatcgtcatc

SEQ ID NO: 64 - DNA, 20 bp, Artificial Sequence
  MMP9_reverse
tcgtcatcgtcgaaatgggc

SEQ ID NO: 65 - DNA, 22 bp, Artificial Sequence
  ACTB_foward
caccattggcaatgagcggttc

SEQ ID NO: 66 - DNA, 22 bp, Artificial Sequence
  ACTB_reverse
aggtctttgcggatgtccacgt

SEQ ID NO: 67 - protein, 710 aa, Artificial Sequence
  VGLL1
METGLGLMETLYSLYSTHRALAILEARGLEPRLYSGLYLYSGLNLYSPRILELYSTHRGLTRPASNSERARGCYSVALLEPHETHRTYRPHEGLNGLYASPILESERSERVALVALASPGLHISPHESERARGALALESERASNILELYSSERPRGLNGLLETHRPRSERSERGLNSERGLGLYVALMETLELYSASNASPASPSERMETSERPRASNGLNTRPARGTYRSERSERPRTRPTHRLYSPRGLNPRGLVALPRVALTHRASNARGALAALAASNCYSASNLEHISVALPRGLYPRMETALAVALASNGLNPHESERPRSERLEALAARGARGALASERVALARGPRGLYGLLETRPHISPHESERSERLEALAGLYTHRSERSERLEGLPRGLYTYRSERHISPRPHEPRALAARGHISLEVALPRGLPRGLNPRASPGLYLYSARGGLPRLELESERLELEGLNGLNASPARGCYSLEALAARGPRGLNGLSERALAALAARGGLASNGLYASNPRGLYGLNILEALAGLYSERTHRGLYLELEPHEASNLEPRPRGLYSERVALHISTYRLYSLYSLETYRVALSERARGGLYSERALASERTHRSERLEPRASNGLTHRLESERGLLEGLTHRPRAGLYLYSTYRSERLEATHRPRAPRAASNHISTRPGLYHISPRAHISARGTYRLEAGLNHISLEA